European Patent Specification EP 4 025 592 B1, published October 29, 2025. Title: CONJUGATED HEPCIDIN MIMETICS. Applicant: Protagonist Therapeutics, Inc. Liu, David Y. Bourne, Gregory Thomas Taranath, Roopa Gupta, Suneel Kumar Modi, Nishit Bachulal. The sequence listing filed with the application follows.

SEQUENCE LISTING (58 sequences)

SEQ ID NO: 1 - protein, 25 aa, Artificial Sequence
  Hepcidin analogue formula
  MOD_RES (1)..(1): Xaa is Asp, Ala, Ida, pGlu, bhAsp, Leu, D-Asp or absent
  MOD_RES (1)..(1): N-terminal residue modified with hydrogen, a C1-C6 alkyl, a C6-C12 aryl, a C1-C20 alkanoyl or pGlu
  MOD_RES (2)..(2): Xaa is Thr, Ala, or D-Thr
  MOD_RES (3)..(3): Xaa is His, Lys or D-His
  MOD_RES (4)..(4): Xaa is Phe, Ala, Dpa or D-Phe
  MOD_RES (5)..(5): Xaa is Pro, Gly, Arg, Lys, Ala, D-Pro or bhPro
  MOD_RES (6)..(6): Xaa is Ile, Cys, Arg, Lys, D-Ile or D-Cys
  MOD_RES (7)..(7): Xaa is Cys, Ile, Leu, Val, Phe, D-Ile or D-Cys
  MOD_RES (8)..(8): Xaa is Ile, Arg, Phe, Gln, Lys, Glu, Val, Leu or D-Ile
  MOD_RES (9)..(9): Xaa is Phe or bhPhe
  MOD_RES (10)..(10): Xaa is Lys, Phe or absent
  MOD_RES (11)..(11): Xaa is Gly, Cys, Ala, Phe, Pro, Glu, Lys, D-Pro, Val, Ser or absent
  MOD_RES (12)..(12): Xaa is Pro, Ala, Cys, Gly or absent
  MOD_RES (13)..(13): Xaa is Arg, Lys, Pro, Gly, His, Ala, Trp or absent
  MOD_RES (14)..(14): Xaa is Ser, Arg, Gly, Trp, Ala, His, Tyr or absent
  MOD_RES (15)..(15): Xaa is Lys, Met, Arg, Ala or absent
  MOD_RES (16)..(16): Xaa is Gly, Ser, Lys, Ile, Ala, Pro, Val or absent
  MOD_RES (17)..(17): Xaa is Trp, Lys, Gly, Ala, Ile, Val or absent
  MOD_RES (18)..(18): Xaa is Val, Thr, Gly, Cys, Met, Tyr, Ala, Glu, Lys, Asp, Arg or absent
  MOD_RES (19)..(19): Xaa is Cys, Tyr or absent
  MOD_RES (20)..(20): Xaa is Met, Lys, Arg, Tyr or absent
  MOD_RES (21)..(21): Xaa is Arg, Met, Cys, Lys or absent
  MOD_RES (22)..(22): Xaa is Arg, Lys, Ala or absent
  MOD_RES (23)..(23): Xaa is Arg, Cys, Lys, Val or absent
  MOD_RES (24)..(24): Xaa is Arg, Lys, Pro, Cys, Thr or absent
  MOD_RES (25)..(25): Xaa is Thr, Arg or absent
  MOD_RES (25)..(25): Xaa is Thr, Arg or absent
  MOD_RES (25)..(25): C-Terminal residue modified with NH2 or OH
XXXXXXXXXXXXXXXXXXXXXXXXX

SEQ ID NO: 2 - protein, 10 aa, Artificial Sequence
  Hepcidin analogue formula
  MOD_RES (1)..(1): Xaa is Asp, Ala, Ida, pGlu, bhAsp, Leu, D-Asp or absent
  MOD_RES (2)..(2): Xaa is Thr, Ala, or D-Thr
  MOD_RES (3)..(3): Xaa is His, Lys or D-His
  MOD_RES (4)..(4): Xaa is Phe, Ala, Dpa or D-Phe
  MOD_RES (5)..(5): Xaa is Pro, Gly, Arg, Lys, Ala, D-Pro or bhPro
  MOD_RES (6)..(6): Xaa is Ile, Cys, Arg, Lys, D-Ile or D-Cys
  MOD_RES (7)..(7): Xaa is Cys, Ile, Leu, Val, Phe, D-Ile or D-Cys
  MOD_RES (8)..(8): Xaa is Ile, Arg, Phe, Gln, Lys, Glu, Val, Leu or D-Ile
  MOD_RES (9)..(9): Xaa is Phe or bhPhe
  MOD_RES (10)..(10): Xaa is Lys, Phe or absent
XXXXXXXXXX

SEQ ID NO: 3 - protein, 15 aa, Artificial Sequence
  Hepcidin analogue formula
  MOD_RES (1)..(1): Xaa is Gly, Cys, Ala, Phe, Pro, Glu, Lys, D-Pro, Val, Ser or absent
  MOD_RES (2)..(2): Xaa is Pro, Ala, Cys, Gly or absent
  MOD_RES (3)..(3): Xaa is Arg, Lys, Pro, Gly, His, Ala, Trp or absent
  MOD_RES (4)..(4): Xaa is Ser, Arg, Gly, Trp, Ala, His, Tyr or absent
  MOD_RES (5)..(5): Xaa is Lys, Met, Arg, Ala or absent
  MOD_RES (6)..(6): Xaa is Gly, Ser, Lys, Ile, Ala, Pro, Val or absent
  MOD_RES (7)..(7): Xaa is Trp, Lys, Gly, Ala, Ile, Val or absent
  MOD_RES (8)..(8): Xaa is Val, Thr, Gly, Cys, Met, Tyr, Ala, Glu, Lys, Asp, Arg or absent
  MOD_RES (9)..(9): Xaa is Cys, Tyr or absent
  MOD_RES (10)..(10): Xaa is Met, Lys, Arg, Tyr or absent
  MOD_RES (11)..(11): Xaa is Arg, Met, Cys, Lys or absent
  MOD_RES (12)..(12): Xaa is Arg, Lys, Ala or absent
  MOD_RES (13)..(13): Xaa is Arg, Cys, Lys, Val or absent
  MOD_RES (14)..(14): Xaa is Arg, Lys, Pro, Cys, Thr or absent
  MOD_RES (15)..(15): Xaa is Thr, Arg or absent
XXXXXXXXXXXXXXX

SEQ ID NO: 4 - protein, 10 aa, Artificial Sequence
  Hepcidin analogue formula
  MOD_RES (1)..(1): Xaa is Asp, Ida, pGlu, bhAsp or absent
  MOD_RES (4)..(4): Xaa is Phe or Dpa
  MOD_RES (5)..(5): Xaa is Pro or bhPro
  MOD_RES (6)..(6): Xaa is Ile, Cys or Arg
  MOD_RES (7)..(7): Xaa is Cys, Ile, Leu or Val
  MOD_RES (8)..(8): Xaa is Ile, Lys, Glu, Phe, Gln or Arg
  MOD_RES (10)..(10): Xaa is Lys or absent
XTHXXXXXFX

SEQ ID NO: 5 - protein, 10 aa, Artificial Sequence
  Hepcidin analogue formula
  MOD_RES (1)..(1): Xaa is Asp, Ida, pGlu, bhAsp or absent
  MOD_RES (4)..(4): Xaa is Phe or Dpa
  MOD_RES (5)..(5): Xaa is Pro or bhPro
  MOD_RES (8)..(8): Xaa is Ile, Lys, Glu, Phe, Gln or Arg
  MOD_RES (10)..(10): Xaa is Lys or absent
XTHXXCIXFX

SEQ ID NO: 6 - protein, 20 aa, Artificial Sequence
  Hepcidin analogue formula
  MOD_RES (1)..(1): Xaa is Asp, Ida, pGlu, bhAsp or absent
  MOD_RES (1)..(1): N-terminal residue modified with hydrogen, isovaleric acid, isobutyric acid or acetyl
  MOD_RES (4)..(4): Xaa is Phe or Dpa
  MOD_RES (5)..(5): Xaa is Pro or bhPro
  MOD_RES (8)..(8): Xaa is Ile, Lys, Glu, Phe, Gln or Arg
  MOD_RES (10)..(10): Xaa is Lys or absent
  MOD_RES (11)..(11): Xaa is Gly, Glu, Val or Lys
  MOD_RES (13)..(13): Xaa is Arg or Lys
  MOD_RES (15)..(15): Xaa is Arg or Lys
  MOD_RES (16)..(16): Xaa is Gly, Ser, Lys, Ile or Arg
  MOD_RES (17)..(17): Xaa is Trp or absent
  MOD_RES (18)..(18): Xaa is Val, Thr, Asp, Glu or absent
  MOD_RES (20)..(20): Xaa is Lys or absent
  MOD_RES (20)..(20): C-terminal residue modified with NH2 or OH
XTHXXCIXFXXPXSXXXXCX

SEQ ID NO: 7 - protein, 10 aa, Artificial Sequence
  Hepcidin analogue formula
  MOD_RES (1)..(1): Xaa is Asp, Ida, pGlu, bhAsp or absent
  MOD_RES (4)..(4): Xaa is Phe or Dpa
  MOD_RES (5)..(5): Xaa is Pro or bhPro
  MOD_RES (8)..(8): Xaa is Ile, Lys, Glu, Phe, Gln or Arg
  MOD_RES (10)..(10): Xaa is Lys or absent
XTHXXCIXFX

SEQ ID NO: 8 - protein, 10 aa, Artificial Sequence
  Hepcidin analogue formula
  MOD_RES (1)..(1): Xaa is Gly, Glu, Val or Lys
  MOD_RES (3)..(3): Xaa is Arg or Lys
  MOD_RES (5)..(5): Xaa is Arg or Lys
  MOD_RES (6)..(6): Xaa is Gly, Ser, Lys, Ile or Arg
  MOD_RES (7)..(7): Xaa is Trp or absent
  MOD_RES (8)..(8): Xaa is Val, Thr, Asp, Glu or absent
  MOD_RES (10)..(10): Xaa is Lys or absent
XPXSXXXXCX

SEQ ID NO: 9 - protein, 18 aa, Artificial Sequence
  Made in Lab - hepcidin peptide analogue
DTHFPICIFGPRSKGWVC

SEQ ID NO: 10 - protein, 19 aa, Artificial Sequence
  Made in Lab - hepcidin peptide analogue
DTHFPCIIFGPRSKGWVCK

SEQ ID NO: 11 - protein, 19 aa, Artificial Sequence
  Made in Lab - hepcidin peptide analogue
DTHFPCIIFEPRSKGWVCK

SEQ ID NO: 12 - protein, 19 aa, Artificial Sequence
  Made in Lab - hepcidin peptide analogue
DTHFPCIIFGPRSKGWACK

SEQ ID NO: 13 - protein, 20 aa, Artificial Sequence
  Made in Lab - hepcidin peptide analogue
DTHFPCIIFGPRSKGWVCKK

SEQ ID NO: 14 - protein, 23 aa, Artificial Sequence
  Made in Lab - hepcidin peptide analogue
DTHFPCIIFVCHRPKGCYRRVCR

SEQ ID NO: 15 - protein, 19 aa, Artificial Sequence
  Made in Lab - hepcidin peptide analogue
DTHFPCIKFGPRSKGWVCK

SEQ ID NO: 16 - protein, 19 aa, Artificial Sequence
  Made in Lab - hepcidin peptide analogue
DTHFPCIKFKPRSKGWVCK

SEQ ID NO: 17 - protein, 19 aa, Artificial Sequence
  Made in Lab - hepcidin peptide analogue
DTHFPCIIFGPRSRGWVCK

SEQ ID NO: 18 - protein, 19 aa, Artificial Sequence
  Made in Lab - hepcidin peptide analogue
DTHFPCIKFGPKSKGWVCK

SEQ ID NO: 19 - protein, 17 aa, Artificial Sequence
  Made in Lab - hepcidin peptide analogue
DTHFPCIKFEPRSKGCK

SEQ ID NO: 20 - protein, 19 aa, Artificial Sequence
  Made in Lab - hepcidin peptide analogue
DTHFPCIKFEPKSKGWECK

SEQ ID NO: 21 - protein, 17 aa, Artificial Sequence
  Made in Lab - hepcidin peptide analogue
DTHFPCIKFEPRSKKCK

SEQ ID NO: 22 - protein, 18 aa, Artificial Sequence
  Made in Lab - hepcidin peptide analogue
DTHFPCIKFEPRSKGCKK

SEQ ID NO: 23 - protein, 17 aa, Artificial Sequence
  Made in Lab - hepcidin peptide analogue
DTHFPCIKFKPRSKGCK

SEQ ID NO: 24 - protein, 17 aa, Artificial Sequence
  Made in Lab - hepcidin peptide analogue
DTHFPCIKFEPKSKGCK

SEQ ID NO: 25 - protein, 9 aa, Artificial Sequence
  Made in Lab - hepcidin peptide analogue
DTHFPCIKF

SEQ ID NO: 26 - protein, 9 aa, Artificial Sequence
  Made in Lab - hepcidin peptide analogue
DTHFPCIIF

SEQ ID NO: 27 - protein, 9 aa, Artificial Sequence
  Made in Lab - hepcidin peptide analogue
DTKFPCIIF

SEQ ID NO: 28 - protein, 19 aa, Artificial Sequence
  Made in Lab - hepcidin peptide analogue
DTHFPCIKFGPRSKGWVCK

SEQ ID NO: 29 - protein, 18 aa, Artificial Sequence
  Made in Lab - hepcidin peptide analogue
DTHFPICIFGPRSKGWVC

SEQ ID NO: 30 - protein, 18 aa, Artificial Sequence
  Made in Lab - hepcidin peptide analogue
DTHFPICIFGPRSKGWVC

SEQ ID NO: 31 - protein, 19 aa, Artificial Sequence
  Made in Lab - hepcidin peptide analogue
DTHFPCIIFGPRSRGWVCK

SEQ ID NO: 32 - protein, 19 aa, Artificial Sequence
  Made in Lab - hepcidin peptide analogue
DTHFPCIIFGPRSRGWVCK

SEQ ID NO: 33 - protein, 19 aa, Artificial Sequence
  Made in Lab - hepcidin peptide analogue
DTHFPCIIFGPRSRGWVCK

SEQ ID NO: 34 - protein, 19 aa, Artificial Sequence
  Made in Lab - hepcidin peptide analogue
DTHFPCIKFGPRSKGWVCK

SEQ ID NO: 35 - protein, 19 aa, Artificial Sequence
  Made in Lab - hepcidin peptide analogue
DTHFPCIKFKPRSKGWVCK

SEQ ID NO: 36 - protein, 19 aa, Artificial Sequence
  Made in Lab - hepcidin peptide analogue
DTHFPCIKFGPKSKGWVCK

SEQ ID NO: 37 - protein, 19 aa, Artificial Sequence
  Made in Lab - hepcidin peptide analogue
DTHFPCIKFGPRSKGWVCK

SEQ ID NO: 38 - protein, 19 aa, Artificial Sequence
  Made in Lab - hepcidin peptide analogue
DTHFPCIKFGPRSKGWVCK

SEQ ID NO: 39 - protein, 19 aa, Artificial Sequence
  Made in Lab - hepcidin peptide analogue
DTHFPCIKFGPRSKGWVCK

SEQ ID NO: 40 - protein, 19 aa, Artificial Sequence
  Made in Lab - hepcidin peptide analogue
DTHFPCIKFKPRSKGWVCK

SEQ ID NO: 41 - protein, 19 aa, Artificial Sequence
  Made in Lab - hepcidin peptide analogue
DTHFPCIKFGPKSKGWVCK

SEQ ID NO: 42 - protein, 19 aa, Artificial Sequence
  Made in Lab - hepcidin peptide analogue
DTHFPCIKFGPRSKGWVCK

SEQ ID NO: 43 - protein, 19 aa, Artificial Sequence
  Made in Lab - hepcidin peptide analogue
DTHFPCIKFGPRSKGWVCK

SEQ ID NO: 44 - protein, 19 aa, Artificial Sequence
  Made in Lab - hepcidin peptide analogue
DTHFPCIKFGPRSKGWVCK

SEQ ID NO: 45 - protein, 17 aa, Artificial Sequence
  Made in Lab - hepcidin peptide analogue
DTHFPCIKFEPRSKGCK

SEQ ID NO: 46 - protein, 17 aa, Artificial Sequence
  Made in Lab - hepcidin peptide analogue
DTHFPCIKFKPRSKGCK

SEQ ID NO: 47 - protein, 17 aa, Artificial Sequence
  Made in Lab - hepcidin peptide analogue
DTHFPCIKFEPKSKGCK

SEQ ID NO: 48 - protein, 17 aa, Artificial Sequence
  Made in Lab - hepcidin peptide analogue
DTHFPCIKFEPRSKGCK

SEQ ID NO: 49 - protein, 18 aa, Artificial Sequence
  Made in Lab - hepcidin peptide analogue
DTHFPCIKFEPRSKGCKK

SEQ ID NO: 50 - protein, 17 aa, Artificial Sequence
  Made in Lab - hepcidin peptide analogue
DTHFPCIKFEPRSKGCK

SEQ ID NO: 51 - protein, 17 aa, Artificial Sequence
  Made in Lab - hepcidin peptide analogue
DTHFPCIKFEPRSKGCK

SEQ ID NO: 52 - protein, 17 aa, Artificial Sequence
  Made in Lab - hepcidin peptide analogue
DTHFPCIKFEPRSKKCK

SEQ ID NO: 53 - protein, 18 aa, Artificial Sequence
  Made in Lab - hepcidin peptide analogue
DTHFPCIKFEPRSKGCKK

SEQ ID NO: 54 - protein, 17 aa, Artificial Sequence
  Made in Lab - hepcidin peptide analogue
DTHFPCIKFEPRSKGCK

SEQ ID NO: 55 - protein, 17 aa, Artificial Sequence
  Made in Lab - hepcidin peptide analogue
  MOD_RES (15)..(15): Xaa is sarcosine
DTHFPCIKFKPRSKXCK

SEQ ID NO: 56 - protein, 25 aa, Homo sapiens
DTHFPICIFCCGCCHRSKCGMCCKT

SEQ ID NO: 57 - protein, 9 aa, Homo sapiens
DTHFPICIF

SEQ ID NO: 58 - protein, 9 aa, Artificial Sequence
  Made in Lab - retro inverse mini hepcidin analogue
  MOD_RES (1)..(1): D form Phe
  MOD_RES (2)..(2): D form Ile
  MOD_RES (3)..(3): D form Cys
  MOD_RES (4)..(4): D form Ile
  MOD_RES (5)..(5): D form Pro
  MOD_RES (6)..(6): D form Phe
  MOD_RES (7)..(7): D form His
  MOD_RES (8)..(8): D form Thr
  MOD_RES (9)..(9): D form Asp
FICIPFHTD